European Patent Specification EP 2 643 348 B1, published February 12, 2025. Title: Improved N-terminal capping modules for designed ankyrin repeat proteins. Applicant: Molecular Partners AG Binz, Hans Kaspar. The sequence listing filed with the application follows.

SEQUENCE LISTING (32 sequences)

SEQ ID NO: 1 - protein, 32 aa, Artificial Sequence
  Synthetic Construct
GSDLGKKLLEAARAGQDDEVRILMANGADVNA

SEQ ID NO: 2 - protein, 28 aa, Artificial Sequence
  Synthetic Construct
QDKFGKTAFDISIDNGNEDLAEILQKLN

SEQ ID NO: 3 - protein, 28 aa, Artificial Sequence
  Synthetic Construct
QDKFGKTPFDLAIREGHEDIAEVLQKAA

SEQ ID NO: 4 - protein, 28 aa, Artificial Sequence
  Synthetic Construct
QDKFGKTPFDLAIDNGNEDIAEVLQKAA

SEQ ID NO: 5 - protein, 32 aa, Artificial Sequence
  Synthetic Construct
  misc_feature (3)..(3): Xaa can be any naturally occurring amino acid
  misc_feature (5)..(5): Xaa can be any naturally occurring amino acid
  misc_feature (21)..(22): Xaa can be any naturally occurring amino acid
  misc_feature (24)..(26): Xaa can be any naturally occurring amino acid
GSXLXKKLLEAARAGQDDEVXXLXXXGADVNA

SEQ ID NO: 6 - protein, 28 aa, Artificial Sequence
  Synthetic Construct
  misc_feature (1)..(1): Xaa can be any naturally occurring amino acid
  misc_feature (4)..(4): Xaa can be any naturally occurring amino acid
  misc_feature (8)..(9): Xaa can be any naturally occurring amino acid
  misc_feature (11)..(13): Xaa can be any naturally occurring amino acid
  misc_feature (15)..(15): Xaa can be any naturally occurring amino acid
  misc_feature (17)..(17): Xaa can be any naturally occurring amino acid
  misc_feature (20)..(20): Xaa can be any naturally occurring amino acid
  misc_feature (23)..(23): Xaa can be any naturally occurring amino acid
XDKXGKTXXDXXXDXGXEDXAEXLQKAA

SEQ ID NO: 7 - protein, 28 aa, Artificial Sequence
  Synthetic Construct
  misc_feature (1)..(1): Xaa can be any naturally occurring amino acid
  misc_feature (4)..(4): Xaa can be any naturally occurring amino acid
  misc_feature (8)..(8): Xaa can be any naturally occurring amino acid
  misc_feature (11)..(13): Xaa can be any naturally occurring amino acid
  misc_feature (15)..(15): Xaa can be any naturally occurring amino acid
  misc_feature (17)..(17): Xaa can be any naturally occurring amino acid
  misc_feature (20)..(20): Xaa can be any naturally occurring amino acid
  misc_feature (23)..(23): Xaa can be any naturally occurring amino acid
XDKXGKTXADXXXDXGXEDXAEXLQKAA

SEQ ID NO: 8 - protein, 28 aa, Artificial Sequence
  Synthetic Construct
  misc_feature (1)..(1): Xaa can be any naturally occurring amino acid
  misc_feature (4)..(4): Xaa can be any naturally occurring amino acid
  misc_feature (8)..(8): Xaa can be any naturally occurring amino acid
  misc_feature (11)..(12): Xaa can be any naturally occurring amino acid
  misc_feature (15)..(15): Xaa can be any naturally occurring amino acid
  misc_feature (17)..(17): Xaa can be any naturally occurring amino acid
  misc_feature (20)..(20): Xaa can be any naturally occurring amino acid
  misc_feature (23)..(23): Xaa can be any naturally occurring amino acid
XDKXGKTXADXXADXGXEDXAEXLQKAA

SEQ ID NO: 9 - protein, 28 aa, Artificial Sequence
  Synthetic Construct
QDKSGKTPADLAADAGHEDIAEVLQKAA

SEQ ID NO: 10 - protein, 33 aa, Artificial Sequence
  Synthetic Construct
  misc_feature (1)..(1): Xaa can be any naturally occurring amino acid
  misc_feature (3)..(4): Xaa can be any naturally occurring amino acid
  misc_feature (6)..(6): Xaa can be any naturally occurring amino acid
  misc_feature (14)..(15): Xaa can be any naturally occurring amino acid
  misc_feature (27)..(27): Xaa can be any naturally occurring amino acid
XDXXGXTPLHLAAXXGHLEIVEVLLKXGADVNA

SEQ ID NO: 11 - protein, 6 aa, Artificial Sequence
  Synthetic Construct
RILLKA

SEQ ID NO: 12 - protein, 6 aa, Artificial Sequence
  Synthetic Construct
RELLKA

SEQ ID NO: 13 - protein, 30 aa, Artificial Sequence
  Synthetic Construct
  misc_feature (1)..(1): Xaa can be any naturally occurring amino acid
  misc_feature (3)..(3): Xaa can be any naturally occurring amino acid
  misc_feature (22)..(22): Xaa can be any naturally occurring amino acid
  misc_feature (24)..(24): Xaa can be any naturally occurring amino acid
XLXKKLLEAARAGQDDEVRILXAXGADVNA

SEQ ID NO: 14 - protein, 32 aa, Artificial Sequence
  Synthetic Construct
GSDLGKKLLEAARAGQDDEVRILLKAGADVNA

SEQ ID NO: 15 - protein, 32 aa, Artificial Sequence
  Synthetic Construct
GSDLGKKLLEAARAGQDDEVRELLKAGADVNA

SEQ ID NO: 16 - protein, 10 aa, Artificial Sequence
  Synthetic Construct
MRGSHHHHHH

SEQ ID NO: 17 - protein, 126 aa, Artificial Sequence
  Synthetic Construct
GSDLGKKLLEAARAGQDDEVRILMKAGADVNAKDEYGLTPLYLATAHGHLEIVEVLLKNGADVNAVDAIGFTPLHLAAFIGHLEIAEVLLKHGADVNAQDKFGKTAFDISIGNGNEDLAEILQKLN

SEQ ID NO: 18 - protein, 126 aa, Artificial Sequence
  Synthetic Construct
GSDLGKKLLEAARAGQDDEVRILLKAGADVNAKDEYGLTPLYLATAHGHLEIVEVLLKNGADVNAVDAIGFTPLHLAAFIGHLEIAEVLLKHGADVNAQDKFGKTAFDISIGNGNEDLAEILQKLN

SEQ ID NO: 19 - protein, 159 aa, Artificial Sequence
  Synthetic Construct
GSDLGKKLLEAARAGQDDEVRILMKAGADVNAFDWMGWTPLHLAAHEGHLEIVEVLLKNGADVNATDVSGYTPLHLAAADGHLEIVEVLLKHGADVNTKDNTGWTPLHLSADLGHLEIVEVLLKNGADVNAQDKFGKTAFDISIDNGNEDLAEILQKLN

SEQ ID NO: 20 - protein, 159 aa, Artificial Sequence
  Synthetic Construct
GSDLGKKLLEAARAGQDDEVRILLKAGADVNAFDWMGWTPLHLAAHEGHLEIVEVLLKNGADVNATDVSGYTPLHLAAADGHLEIVEVLLKHGADVNTKDNTGWTPLHLSADLGHLEIVEVLLKNGADVNAQDKFGKTAFDISIDNGNEDLAEILQKLN

SEQ ID NO: 21 - protein, 93 aa, Artificial Sequence
  Synthetic Construct
GSDLGKKLLEAARAGQDDEVRILMANGADVNAKDKDGYTPLHLAAREGHLEIVEVLLKAGADVNAQDKFGKTAFDISIDNGNEDLAEILQKLN

SEQ ID NO: 22 - protein, 93 aa, Artificial Sequence
  Synthetic Construct
GSDLGKKLLEAARAGQDDEVRILLAAGADVNAKDKDGYTPLHLAAREGHLEIVEVLLKAGADVNAQDKFGKTAFDISIDNGNEDLAEILQKLN

SEQ ID NO: 23 - protein, 93 aa, Artificial Sequence
  Synthetic Construct
GSDLGKKLLEAARAGQDDEVRILLKAGADVNAKDKDGYTPLHLAAREGHLEIVEVLLKAGADVNAQDKFGKTAFDISIDNGNEDLAEILQKLN

SEQ ID NO: 24 - protein, 126 aa, Artificial Sequence
  Synthetic Construct
GSDLGKKLLEAARAGQDDEVRILMANGADVNAKDYFSHTPLHLAARNGHLKIVEVLLKAGADVNAKDFAGKTPLHLAANDGHLEIVEVLLKHGADVNAQDIFGKTPADIAADAGHEDIAEVLQKLN

SEQ ID NO: 25 - protein, 126 aa, Artificial Sequence
  Synthetic Construct
GSDLGKKLLEAARAGQDDEVRILLKAGADVNAKDYFSHTPLHLAARNGHLKIVEVLLKAGADVNAKDFAGKTPLHLAANDGHLEIVEVLLKHGADVNAQDIFGKTPADIAADAGHEDIAEVLQKLN

SEQ ID NO: 26 - protein, 126 aa, Artificial Sequence
  Synthetic Construct
GSDLGKKLLEAARAGQDDEVRELLKAGADVNAKDYFSHTPLHLAARNGHLKIVEVLLKAGADVNAKDFAGKTPLHLAANDGHLEIVEVLLKHGADVNAQDIFGKTPADIAADAGHEDIAEVLQKLN

SEQ ID NO: 27 - protein, 126 aa, Artificial Sequence
  Artificial Sequence
GSDLGKKLLEAARAGQDDEVRILMANGADVNAADYFSHTPLHLAARNGHLKIVEVLLKYGADVNASDFAGKTPLHLAANDGHLEIVEVLLKHGADVNAQDIFGKTAFDISIDNGNEDLAEILQKLN

SEQ ID NO: 28 - protein, 126 aa, Artificial Sequence
  Synthetic Construct
GSDLGKKLLEAARAGQDDEVRILMANGADVNAADYFSHTPLHLAARNGHLKIVEVLLKYGADVNASDFAGKTPLHLAANDGHLEIVEVLLKHGADVNAQDIFGKTPADIAADNGHEDIAEVLQKLN

SEQ ID NO: 29 - protein, 126 aa, Artificial Sequence
  Synthetic Construct
GSDLGKKLLEAARAGQDDEVRILLAAGADVNAADERGTTPLHLAAVYGHLEIVEVLLKNGADVNAQNETGYTPLHLADSSGHLEIVEVLLKHSADVNAQDKFGKTAFDISIDNGNEDLAEILQKLN

SEQ ID NO: 30 - protein, 126 aa, Artificial Sequence
  Synthetic Construct
GSDLGKKLLEAARAGQDDEVRILLAAGADVNAADERGTTPLHLAAVYGHLEIVEVLLKNGADVNAQNETGYTPLHLADSSGHLEIVEVLLKHSADVNAQDKSGKTPADIAADNGHEDIAEVLQKLN

SEQ ID NO: 31 - protein, 103 aa, Artificial Sequence
  Synthetic Construct
MRGSHHHHHHGSDLGKKLLEAARAGQDDEVRILMANGADVNAKDKDGYTPLHLAAREGHLEIVEVLLKAGADVNAQDKFGKTAFDISIDNGNEDLAEILQKLN

SEQ ID NO: 32 - protein, 103 aa, Artificial Sequence
  Synthetic Construct
MRGSHHHHHHGSDLGKKLLEAARAGQDDEVRILMANGADVNAKDKDGYTPLHLAAREGHLEIVEVLLKAGADVNAQDKSGKTPADLAADNGHEDIAEVLQKAA